European Patent Specification EP 4 392 177 B1, published April 23, 2025. Title: Detection of SARS-CoV-2. Applicant: MIP Discovery Limited. Application EP. The sequence listing filed with the application follows.

SEQUENCE LISTING (9 sequences)

SEQ ID NO: 1 - protein, 11 aa, Severe acute respiratory syndrome-related coronavirus
NSNNLDSKVGG

SEQ ID NO: 2 - protein, 12 aa, Severe acute respiratory syndrome-related coronavirus
NYNYLYRLFRKS

SEQ ID NO: 3 - protein, 12 aa, Severe acute respiratory syndrome-related coronavirus
YRLFRKSNLKPF

SEQ ID NO: 4 - protein, 12 aa, Severe acute respiratory syndrome-related coronavirus
STEIYQAGSTPC

SEQ ID NO: 5 - protein, 11 aa, Severe acute respiratory syndrome-related coronavirus
CNGVEGFNCYF

SEQ ID NO: 6 - protein, 11 aa, Severe acute respiratory syndrome-related coronavirus
GSTPCNGVEGF

SEQ ID NO: 7 - protein, 12 aa, Severe acute respiratory syndrome-related coronavirus
CYFPLQSYGFQP

SEQ ID NO: 8 - protein, 11 aa, Severe acute respiratory syndrome-related coronavirus
GFQPTNGVGYQ

SEQ ID NO: 9 - protein, 11 aa, Severe acute respiratory syndrome-related coronavirus
LQSYGFQPTNG